European Patent Application EP 4 527 919 A1, published March 26, 2025. Title: Prevotella histicola. Applicant: Kookmin University Industry Academy Cooperation Foundation. Application KR. The sequence listing filed with the application follows.

SEQUENCE LISTING (5 sequences)

SEQ ID NO: 1 - DNA, 20 bp, synthetic construct
  misc_feature 1..20: note = universal PCR primer 27F
  variation 12: note = M is A or C
  source 1..20: mol_type = other DNA
agagtttgatcmtggctcag

SEQ ID NO: 2 - DNA, 22 bp, synthetic construct
  misc_feature 1..22: note = universal PCR primer 1492R
  variation 6: note = Y is C or T
  source 1..22: mol_type = other DNA
tagggytaccttgttacgactt

SEQ ID NO: 3 - DNA, 1452 bp, synthetic construct
  misc_feature 1..1452: note = Prevotella histicola KCOM 3796 16S rDNA
  source 1..1452: mol_type = other DNA
gatgaacgctagctacaggcttaacacatgcaagtcgaggggaaacggcattaagtgcttgcactttttggacgtcgaccggcgcacgggtgagtaacgcgtatccaaccttcccatgactaagggataacctgccgaaaggcagactaataccttatggtcttcactgacggcatcagatgtgaagtaaagatttatcggttatggatggggatgcgtctgattagcttgttggcggggtaacggcccaccaaggcaacgatcagtaggggttctgagaggaaggtcccccacattggaactgagacacggtccaaactcctacgggaggcagcagtgaggaatattggtcaatgggcgagagcctgaaccagccaagtagcgtgcaggatgacggccctatgggttgtaaactgcttttgtatggggataaagtcaatcacgtgtgattgtttgcaggtaccatacgaataaggaccggctaattccgtgccagcagccgcggtaatacggaaggtccgggcgttatccggatttattgggttaaagggagcgtaggctggagattaagtgtgttgtgaaatgtagacgctcaacgtctgacttgcagcgcatactggtttccttgagtacgcacaacgttggcggaattcgtcgtgtagcggtgaaatgcttagatatgacgaagaactccgattgcgaaggcagctgacgggagcgcaactgacgctgaagctcgaaggtgcgggtatcgaacaggattagataccctggtagtccgcacagtaaacgatggatgcccgctgttggtacgtggtatcagcggctaagcgaaagcattaagcatcccacctggggagtacgccggcaacggtgaaactcaaaggaattgacgggggcccgcacaagcggaggaacatgtggtttaattcgatgatacgcgaggaaccttacccgggcttgaattgcagaggaaggatttagagataatgacgcccttcggggtctctgtgaaggtgctgcatggttgtcgtcagctcgtgccgtgaggtgtcggcttaagtgccataacgagcgcaacccctgtctttagttgccatcaggtgatgctgggcactctggagatactgccaccgtaaggtgtgaggaaggtggggatgacgtcaaatcagcacggcccttacgtccggggctacacacgtgttacaatggccggtacagagggacggtgtaatgtaaattgcatccaatcttgaaagccggtcccagttcggactggggtctgcaacccgaccccacgaagctggattcgctagtaatcgcgcatcagccatggcgcggtgaatacgttcccgggccttgtacacaccgcccgtcaagccatgaaagccgggggtgcctgaagtccgtgaccgcaaggatcggcctagggcaaaactggtgattggggct

SEQ ID NO: 4 - DNA, 1453 bp, synthetic construct
  misc_feature 1..1453: note = Prevotella histicola KCOM 4081 16S rDNA
  source 1..1453: mol_type = other DNA
gatgaacgctagctacaggcttaacacatgcaagtcgaggggaaacggcattaagtgcttgcactttttggacgtcgaccggcgcacgggtgagtaacgcgtatccaaccttcccatgactaagggataacctgccgaaaggcagactaataccttatggtcttcactgacggcatcagatgtgaagtaaagatttatcggttatggatggggatgcgtctgattagcttgttggcggggtaacggcccaccaaggcgacgatcagtaggggttctgagaggaaggtcccccacattggaactgagacacggtccaaactcctacgggaggcagcagtgaggaatattggtcaatgggcgagagcctgaaccagccaagtagcgtgcaggatgacggccctatgggttgtaaactgcttttgtatggggataaagtcaatcacgtgtgattgtttgcaggtaccatacgaataaggaccggctaattccgtgccagcagccgcggtaatacggaaggtccgggcgttatccggatttattgggtttaaagggagcgtaggctggagattaagtgtgttgtgaaatgtagacgctcaacgtctgacttgcagcgcatactggtttccttgagtacgcacaacgttggcggaattcgtcgtgtagcggtgaaatgcttagatatgacgaagaactccgattgcgaaggcagctgacgggagcgcaactgacgctgaagctcgaaggtgcgggtatcgaacaggattagataccctggtagtccgcacagtaaacgatggatgcccgctgttggtacctggtatcagcggctaagcgaaagcattaagcatcccacctggggagtacgccggcaacggtgaaactcaaaggaattgacgggggcccgcacaagcggaggaacatgtggtttaattcgatgatacgcgaggaaccttacccgggcttgaattgcagaggaaggatttagagataatgacgcccttcggggtctctgtgaaggtgctgcatggttgtcgtcagctcgtgccgtgaggtgtcggcttaagtgccataacgagcgcaacccctgtctttagttgccatcaggtgatgctgggcactctggagatactgccaccgtaaggtgtgaggaaggtggggatgacgtcaaatcagcacggcccttacgtccggggctacacacgtgttacaatggccggtacagagggacggtgtaatgtaaattgcatccaatcttgaaagccggtcccagttcggactggggtctgcaacccgaccccacgaagctggattcgctagtaatcgcgcatcagccatggcgcggtgaatacgttcccgggccttgtacacaccgcccgtcaagccatgaaagccgggggtgcctgaagtccgtgaccgcaaggatcggcctagggcaaaactggtgattggggct

SEQ ID NO: 5 - DNA, 1453 bp, synthetic construct
  misc_feature 1..1453: note = Prevotella histicola KCOM 4227 16S rDNA
  source 1..1453: mol_type = other DNA
gatgaacgctagctacaggcttaacacatgcaagtcgaggggaaacggcattaagtgcttgcactttttggacgtcgaccggcgcacgggtgagtaacgcgtatccaaccttcccatgactaagggataacctgccgaaaggcagactaataccttatggtcttcactgacggcatcagatgtgaagtaaagatttatcggttatggatggggatgcgtctgattagcttgttggcggggtaacggcccaccaaggcaacgatcagtaggggttctgagaggaaggtcccccacattggaactgagacacggtccaaactcctacgggaggcagcagtgaggaatattggtcaatgggcgagagcctgaaccagccaagtagcgtgcaggatgacggccctatgggttgtaaactgcttttgtatggggataaagtcaatcacgtgtgattgtttgcaggtaccatacgaataaggaccggctaattccgtgccagcagccgcggtaatacggaaggtccgggcgttatccggatttattgggtttaaagggagcgtaggctggagattaagtgtgttgtgaaatgtagacgctcaacgtctgacttgcagcgcatactggtttccttgagtacgcacaacgttggcggaattcgtcgtgtagcggtgaaatgcttagatatgacgaagaactccgattgcgaaggcagctgacgggagcgcaactgacgctgaagctcgaaggtgcgggtatcgaacaggattagataccctggtagtccgcacagtaaacgatggatgcccgctgttggtacttggtatcagcggctaagcgaaagcattaagcatcccacctggggagtacgccggcaacggtgaaactcaaaggaattgacgggggcccgcacaagcggaggaacatgtggtttaattcgatgatacgcgaggaaccttacccgggcttgaattgcagaggaaggatttagagataatgacgcccttcggggtctctgtgaaggtgctgcatggttgtcgtcagctcgtgccgtgaggtgtcggcttaagtgccataacgagcgcaacccctgtctttagttgccatcaggttaagctgggcactctggagatactgccaccgtaaggtgtgaggaaggtggggatgacgtcaaatcagcacggcccttacgtccggggctacacacgtgttacaatggccggtacagagggacggtgtaatgtaaattgcatctaatcttgaaagccggtcccagttcggactggggtctgcaacccgaccccacgaagctggattcgctagtaatcgcgcatcagccatggcgcggtgaatacgttcccgggccttgtacacaccgcccgtcaagccatgaaagccgggggtgcctgaagtccgtgaccgcaaggatcggcctagggcaaaactggtgattggggct